European Patent Specification EP 3 568 145 B1, published June 11, 2025. Title: MATERIALS AND METHODS FOR TREATING CANCER. Applicant: Mayo Foundation for Medical Education and Research. The sequence listing filed with the application follows.

SEQUENCE LISTING (3 sequences)

SEQ ID NO: 1 - DNA, 16 bp, Artificial Sequence
  synthetic primer
gggtgtgccggttgga

SEQ ID NO: 2 - DNA, 22 bp, Artificial Sequence
  synthetic primer
agaagccagggagagctacaga

SEQ ID NO: 3 - DNA, 23 bp, Artificial Sequence
  synthetic probe
tgggcagctctcgcatcacttgc